European Patent Application EP 4 560 016 A1, published May 28, 2025. Title: Method of plant genome editing. Applicant: Plantik Biosciences. Application EP. The sequence listing filed with the application follows.

SEQUENCE LISTING (4 sequences)

SEQ ID NO: 1 - DNA, 20 bp, synthetic construct
  source 1..20: mol_type = other DNA
agggagctggcagagcatcg

SEQ ID NO: 2 - DNA, 20 bp, synthetic construct
  source 1..20: mol_type = other DNA
caatgcccagcaagccagga

SEQ ID NO: 3 - DNA, 21 bp, synthetic construct
  source 1..21: mol_type = other DNA
cggtgactggtatgagaccgg

SEQ ID NO: 4 - DNA, 23 bp, synthetic construct
  source 1..23: mol_type = other DNA
caggtcagcatctcattgttccg